European Patent Specification EP 3 820 909 B1, published March 1, 2023. Title: MONOCLONAL ANTIBODY FOR THE DETECTION OF THE ANTIRETROVIRAL DRUG EMTRICITABINE (FTC, 2',3'-DIDEOXY-5-FLUORO-3'-THIACYTIDINE). Applicant: THE UNITED STATES OF AMERICA, as represented by the Secretary, Department of Health and Human Services Granade, Timothy C Youngpairoj, Ae S Switzer, William M Heneine, Walid M Pau, Chou-Pong Zheng, HaoQiang Pohl, Jan. The sequence listing filed with the application follows.

SEQUENCE LISTING (8 sequences)

SEQ ID NO: 1 - protein, 456 aa, Mus musculus
QVQLQQPGAELVKPGASVKVSCKASGYTFTSYWMHWVKQRPGQGLEWIGRIHLSDSDTNYNQNFKDKATLTVDKSSRTAHMHLSSLTSADSAVYYCAMGGTFQSNYDTYWGQGTLVTVSAAKTTPPSVYPLAPGCGDTTGSSVTLGCLVKGYFPESVTVTWNSGSLSSSVHTFPALLQSGLYTMSSSVTVPSSTWPSQTVTCSVAHPASSTTVDKKLEPSGPISTINPCPPCKECHKCPAPNLEGGPSVFIFPPNIKDVLMISLTPKVTCVVVDVSEDDPDVRISWFVNNVEVHTAQTQTHREDYNSTIRVVSALPIQHQDWMSGKEFKCKVNNKDLPSPIERTISKIKGLVRAPQVYILPPPAEQLSRKDVSLTCLVVGFNPGDISVEWTSNGHTEENYKDTAPVLDSDGSYFIYSKLDIKTSKWEKTDSFSCNVRHEGLKNYYLKKTISRSPGK

SEQ ID NO: 2 - protein, 214 aa, Mus musculus
DIQMTQSPASLSASVGETVTITCRASGNIHNYLAWYQQKQGKSPQLLVYNAKTLTDGVPSRFSGSGSGTQYSLKINSLQPEDFGNYYCQHFLYTPYTFGGGTKLEMRRADAAPTVSIFPPSSEQLTSGGASVVCFLNNFYPKDINVKWKIDGSERQNGVLNSWTDQDSKDSTYSMSSTLTLTKDEYERHNSYTCEATHKTSTSPIVKSFNRNEC

SEQ ID NO: 3 - DNA, 317 bp, Mus musculus
gggcttcagtgaaggtgtcctgcaaggcatctggctacaccttcaccagctactggatgcactgggtgaagcagaggcctggccaaggccttgagtggattggaaggattcatctttctgatagtgatactaactacaatcaaaacttcaaggacaaggccacattgactgtagacaaatcctcccgcacagcccacatgcatctcagcagcctgacatctgcggactctgcggtctattattgtgcaatgggggggaccttccagagtaactacgatacttactggggccaagggactctggtcactgtctctgca

SEQ ID NO: 4 - DNA, 381 bp, Mus musculus
atgagtgtgctcactcaggtcctggcgttgctgctgctgtggcttacaggtgccagatgtgacatccagatgactcagtctccagcctccctatctgcatctgtgggagaaactgtcaccatcacatgtcgagcaagtgggaatattcacaattatttagcatggtatcagcagaaacagggaaaatctcctcagctcctggtctataatgcaaaaaccttaacagatggtgtgccatcaaggttcagtggcagtggatcaggaacacaatattctctcaagatcaacagcctgcagcctgaagattttgggaattattactgtcaacattttttgtatactccttacacgttcggaggggggaccaagctggaaatgaga

SEQ ID NO: 5 - protein, 19 aa, Artificial Sequence
  Leader
MRWSCLILFLLATTPGVHS

SEQ ID NO: 6 - protein, 120 aa, Mus musculus
QVQLQQPGAELVKPGASVKVSCKASGYTFTSYWMHWVKQRPGQGLEWIGRIHLSDSDTNYNQNFKDKATLTVDKSSRTAHMHLSSLTSADSAVYYCAMGGTFQSNYDTYWGQGTLVTVSA

SEQ ID NO: 7 - protein, 20 aa, Artificial Sequence
  Leader
MSVLTQVLALLLLWLTGARC

SEQ ID NO: 8 - protein, 107 aa, Mus musculus
DIQMTQSPASLSASVGETVTITCRASGNIHNYLAWYQQKQGKSPQLLVYNAKTLTDGVPSRFSGSGSGTQYSLKINSLQPEDFGNYYCQHFLYTPYTFGGGTKLEMR